European Patent Application EP 4 137 568 A1, published February 22, 2023. Title: Novel polypeptides and antibiotics against Gram-negative bacterium comprising the same. Applicant: LyseNTech Co., Ltd. Application EP, filed August 19, 2022. The sequence listing filed with the application follows.

SEQUENCE LISTING (13 sequences)

SEQ ID NO: 1 - DNA, 42751 bp, synthetic construct
  misc_feature 1..42751: note = synthetic_Bacteriophage EC340-M-11-12 whole genome
  source 1..42751: mol_type = other DNA
gttctcgtcggtagatgtgtcggtgttcgatggctccacgccgttgcgttgcgatactctcaccatcaccaacgacaacggagcttccgcgcagttcgaactcggtaacagtagcgtggcgttcgtcgaacgtggacgcgcagctaacacattctctatctctggcaagctgtacgacatggcgatgattcagaagtttatcaacgagcagcaggtagagattaactctattctggcaggggtaaacggggctatgtctttcagtttgaaacgtgcagagcttacggcggttacacctgagattggtgggcctgagtcaatcactcagtccattgaaggccaggctaccggcaatcagtaccagtcgtctatcgtaattcaacgtatcacctacgcataaaactaaggcccctttcggggcctttttcttacaaacctaattttaaagcaatgtctataacgttcgatttaacgtcacccggtatgatgtaggtgtcgtaatcttttacaccactaacatcgtacagatagccacggctatcgcagatgaacgtatagccgtcacgatggaggcggacgattcgcacgtcatgccccgcggcgacgataggggcaacttcactggcgaatccaccatcggacactacaaaaacttcgtcgccgtcaggcaagttttcagcaagatacttaccgaaataatcatcgccgaataccggtttaatgaattgctcagaaatggcaatcattaaccggcggcgggacaacccattaagaaaaccctcgggtttttctttccgcgcccggtcgtcgtagccgtcgagaaattcgtggtaagcatcctggcctaacgctgccaaagcaatattgaacattggattcttgaaactggtagttcctttcgcaaagcccatttctaccagcgccatagcaagcgtgtctttcccgcaacccgcagggccattaagaataattaccttagccattatttatcgctccagtgtggttttaagtgtgtagagttcccgttacagtcgtattcggtaactgcgtgtgcggttatgccgaggtcacggaaatgctttattaccgctggggagtcgtcgaacgcacacaagattctttccagtccgaaagcacgcaacacctcttctttaattacgatgtcttttctgttgtcgtgtttgctgcgcatgattagcgtgtcaaacctaacgttattctctcgtaaccattcgcgagtctcctcctcagcgtcatcacttcgcccggtaaggataattatagtaagtccggaatgccacagtacgctacacaaatggatattgtcgtatatcggagcgtcatctttgcaggccatgttaaatggcttccacgcccacgtttctccgtagttatcttttggtaacaggtgtaagcgatgggtaccgtcggccaatgtcccgtctaaatcgaaaattacaatatctttcatcccagcatctccggtgaaatagttaaacgtgcgacctcgccatattcggcgctataagtaattacatttgcactgcggcccgacatccatccgccgcgagaggcgtaggcgtctttagccgctaaggtgcggtgttgctcaacaatcatgttacggctttctacaatcttctggtggtgcagatggcctacgtgggcgtagctgtaaacactctcgccgaacgctttacggaacttggcaatcataaccggttcgatagcgtcgaatcgtgctttatgcccgtgatggaagaacagcgtcgttttgccgtgttgcaccatcttgtaaacatccggcgacgtatcaacaatcactcggctgtcgtttgagtataaaaccgtgaacatttcggcaagccatacggagccaacagggtcgtggttaccttgaacgattaaaagttttactgtgtgatgcttaaccagcgccatatcaacaacacggcggaccatacgaatcatgtaacgtaccagtttctgatagcgagtatccgcatctaatacatggcgcgactcgggggtaacggcatcaagactatcgaagtgtgcgaagtccccaagcaggttaataactcctgttcctgcatccggtgctttctgaaacgccgcgtcgaaccaccgagagaacaggtcttctgcaatcttcatgtcccagtcgtcgccgctctcatcggcccatgccagcataccgagatggaaatcagatacagtgtaaagattgagtagcttgtcgtcacgtttggcgcgcgccgctttaacaggcgcaacgggcgtaatctctgacttcatgccctctattacggctttcatcaattcaacctgacgttcggcgtcggtgtctgtcttaacccactgcaacttagtgttaccgaactcgtccaccagagacgacgtgcctttaatcttgtagccgtctggtacaaggtggcttacgtcccgcccgtggcctacgcctttcttagccagcttcgctttacggattcggataacgcggtctgagattccgtatttacgggcgatatcgatattcttcatcccggcgttcaattcttcctgtaattgctcgtcggttattttcttctgggccatgcttacttcctcgtgtttaggatttgtcttatagtagcctacttctctttcacgttcgagttgcaagcccagattaaaatgaatacccacggcaacagaatccacccgagaaataagttagccatgaatatcgccagctttgctttatggttacgcatatgtgccaccaaaaacgggataaaataaacggctacaaaaataattaagaagaacatagtgataccggtcataacataactcctgatttgagataacatcgttggtgtaagtgaatagtacgctattatattggggtgtgcaagtagtgtgctagaataattttgcgcctagtgtcgcacacgaaaagcgggtggttcccgtctggcgcatttcctttaaccagtaacctcttaaccaaaggattaaagaatgaaactttctgatttttattacgaagcggaagccgaaaagggcgcacgtatgccgataccgctaaaagacggtactgattccggggaatggcttaatgttgtttctcctgaggcggacgttgccgttaaggctatgcgcgcgttcacccttgcataccgggcagtattagggaaattaaaaccgcttcgtgataagtgcgaagagatgaaagatttctctgaatacaacctgaagatggaagacgcggcgacggaccttaaccgtcagttagcgattgaattggttaacgggtggagccttgacgacgaattcaataaagagaatctgaacacactcctgacgcaatataaacgactcgcggaacttgttgttgtgtttcataacgaacaactgcaccagctacaggaaaagtagacgcgttgctccagttcgcccgttggaacttcataacccgccacaaacggcgggaatttgacagtatcgccgatgggcataaagccgcgctaattgctatgggggttatgcaagacgcgccggatgcaacgcaggccgctgggccggaatgcccccctgagctactaaccacatttgagaagtacagggaaattaaattcacccgccgagtggacgacgacggcatcaagatgtacccgcgcgagcaattacgatggtcagatttagtggcgtacagcaccgtttcaggccagaatatagggatgttcgaatccgacatcatcatgagcttagacgctattttcgagggtagaaacgatggctgatgtagctagtttagtagtaaaagtaacagagcaaggcgcgaaagccacatcagaccgtcttgacaacctttcaaagtccgcaaaagtagcgggggccgccgtagcaggccttgcttctatcgtagcggctaccgcgtataaagctgcccaagaactggttgactcacagcggcaactggacaagatgtccgccagtttgaagaccttaacaggaagtacccaaggtgctaaacaggcgctaagtatcctgcaagattttgcccgcgataccccatacggactggagcaggcggtggaaggcttccgtaagctggtggcccttggccttaccccatccgaggaggcgttgcggtcctacggcaataccgcatcggctatgggcaaggaccttaatcagatgattgaggcggtagccgacgccagtacgtttgagttcgaacgcctaaaagaattcggcatcaaagccaagcagaacaaaaacgacgtagagtttacattccaggggacaacaaccgtagttaagaaaagcgctgccgatattgagcagtatttacttaatattggtaacgtaaattttgccggtgccatggcggaccaggccaacacccttaatggtgctatcgcgagcgccagtgactcatggtcgcagctaaaaatgacgcttgccaccagtcttgatgttggcgcacttgcggaacctatcaggtatatcgatgacttgatccaggaattaaacgcgtctgttgcttccggtgaattagccgctgaaatgcagatgtggggcgacatagcgtcggaagtaggaagcgctatcgagatgtcattcgacgctgcgtttggctttgttggtgatgccatcaacgggcttaatgaactgtgggatttcagcagcaagagtattaccgatagcggagaacaaacggccaccaccatcgctgaatccgccgccgatgctcttgacttcatcgcggaagagttcaccgcgatggagagattctttgaagatatggttaaaggtgctcaggacgctggccgtcttgtacgcgccgcttttacccccggggaatcagtagacgtagctaaaaatatcaacttccagcttggcatggctttggatacccagcgcgatgtcgccgacgttacgcgtaaaagtttccgcgaacaggtagaagctcaacaggatattgtagcgttaaaacgcgcggcgtatgacatcgataaggagtccgcaaaagctgaggggttaaacaaatttaaggtaaccggaaccggcggcggttctgacgatgacgggtcagccgcaaaagccgctaagaaagcagcggacgcgttcgagcgccagaaaaaggcggcggaagacttctactatcagtcaatccatcttaatgatgacgtatttcagaaaatagaagctaaccaggaagagcaactgtctaagttgcaggatttttatagcaataagcttcttagcgaccaacagtacgaaaacgccaagacgcagattatgctctctgccgaacaggcccgccaggaagaactggacaagaaaaggaaagaagcccaggagaagcagcagaaaggtgatgatttcatggctcagattatgggccagaacgccaccgagcttgagcttctggatattcaggaacagcagaaactggcggtagccgataagtaccgggaacaaggtctgattagcgagaagcagtatcaggccgcgcttaacgccatcaacgagcagtacgcaaccaagcgtgccgacgcaacggcaacagctttcggtaacatggcctcaaacatcgggtctgcgttgggcgaggcttctggcgcgtataaagcattcgctatcgtacaggctactatagccacgtacaccgcagctattgaggcatacaagtcaacggcggctatccctgtagtcggtccgttcctggccccagtagccgctgctgctgctgttggggccggtatggcgcaggtttccgctatcaggtccgcgcgtgaacagggcggtcagttatcagcaggacaggcttcaaccatcgccgaacgcggtaaaccagaagttatcatgcccgctggtgcgtcacgtgtacgcaccgcacagcagatgaaagaaattatggggcaaaacgggtcttcttccggaccgtctaatgttactatcgtaaacaacacgagttctcaaatcggcaacgtatccactgagcaagatgatgaaggccgtttgcgtatcatcatcgaggagcaagtggctgcctctttgcagaacagtaacagtaagattagcaaggcccgcaaggccacaagaaatgcgccggggtttaaataatgagcgacttatatttcccacgtagccttaagccggtggtatcgaaaggctactcaatgaccagacgcaacaacgtctggagtgtagatttagccggtggcggagtgcgtcaaggccgtgacacgtattatgatgtgttcccaataagcgtaaccctgattacatccgcaatggggcggcaggcgtttctgtcgttcctcgagaaagtcgatggtggcgcgtcaagtttctggatggcgcacgacttcggcatgggtattgaggattatcaagtcaccattacatccaccgtcgccgagtccactgaagacgggattaactggacaattactttcacggcaaccgctgagaaatcaccgttccaggacctcgagaaccagtgccttgttaacaatctgccggatttgtatggttgttatggtgacgggctggggtgtatccttaaagcctacggaaccgcacaatcaacgtttccacgaatttgggaaccgatgcaatgagccaggaatctgtagaagccgcctatcgccgtaagctggcctcaaatcccgacggcgagatggattacatcacattgcaaatcagccacccgttgttgtcaaagacgtactatcttgtgcgcgggttacaggaactcacggcaacactggagacaggcgaaattatcacgttcgagccaaccccgatggaggcgtcgggggcggctaacaacagtgatatggaccagacgactacgtttactttaccggatattctcaatcaacttgacgatgagatggataaaatccctatgagtaacaccgagttgccgaagttcgtcttccgtcgttacgtcagcacagacctgtcttatccggctgacggtcctgtcatgtatgagttgcaggccatcaaccaggagaagggcgagttctccgcggatgttggtacacctatgctgaaccagcgaagcactggtatactgatgacacctaaagagataccgttattacgcggcctgttgaccacatgaatattaacgactacacgggcataccttacgactttcgcaagcgcaattgctggcatcacgtgcgcattgtccgcgcggatgccgggttagaaacccctgcgttcgacgttacaagcccatcggcaattaacgaagcgtttgacgaaggccaccgtgacacgaaggggcttacaaaaattgataagcctgaaaacttctgcgcggtgcttatgggttatcgtcgcgggggtcgtatcgtgtggcacgctggagtttacttcgacgggatggtgagtcattgcgagcttgcatcccgtcaggtacggcttgacaggctggtggacctcagagacacgtacacggagattgaattttggcgataatcctgcactacacgcgaaacgctgaaggcgctttcgaccgtacaaaacacgtcgggatgccgatggagtttgtcgttaaccgtattccctacggcgtgcctgtgcgcgtctatctcggtgagattggcgatgatacagatgtaacagacgacttcaatgcgctcaaagacgaggacgccgtgtaccacattatcgagggtgcaggcggtggtatcggcgacgctatcggtagtgtattcagtttcatccttaagccaattgccaaattgttcgggctaaacacagcagctaacgctaattattccgctaccaacaatcaggctacgtcgcctaacaacagtcttactgaccgctcgaacaagccacgtccttatgaacgttcttatgacatctgcgggacagtgcagactatacccaatgacctgatgcagacgtataaggtgtttaacgccacgggggcgcttattgaatatgcgtactatgacgccggtcgagggtatctgcatattgaggaagacggtgtaactgaggcagatacccgaatcagcgagataactggctcgtcggtgacggtgtattctccttacacttcgccgaataacaccagcacaccacaattgcatatcggcgaccctatagaccagaaattgtacgttacatttaaaaacgccgatgtcgatggcgctgttcttcccgcccctaatgatatcgctatagacgtgcaggactacactgtccagcggcagggaacaaccggcgttgtagtaggcgatgacgctggtttcgatgagtttttggcggtcggggacctggcatacttcgataacgtatatgcagatacaaccccagggtctttgggtaatgaggttaacctggacgggaggtacacggttctttctgttagtgaaacgacccttattgtggacgtcagtacaaatcaatcaatatggaaccagctaggaacatctgtatggtttataggtgaagagggcaaccatcttataggcccggcggatacttacgcggcttccctctctgaatgggcgtacatcacccgcggaaccgtcgaccgtgttgtagccaatgtggctgccagcaacggcatgtacaaatacaacggcgactataaccgcgcttcagtgacagtcgaactgcaataccagatggtagatgaattgaaacagcctgtaggtgacatatttaccgtacgaggaaccgtaacaggccggaacacggattacacagggattactctttacggaagtttaccaactgcttccagattccgcgcccgtatgcgtcgtgtttcggacaccgataaagattttgaaggtactgttagcgacgaggttactttcactaatctgtatgggcagtcgctggacacaaccccccactacggcaaccgtactaccgtacactgcgcccgtaaacaaaccccacgtgcagccgaggtgtccgaaccggaactgcgcatgattgcaaccgagatgtgctacaaatacttaggtaacggcgtattcgatacggtaatgacaccgaacactcaggccgtgcagtcgctaatcaggctggcgcgtgaccctgtggtgggtaatctggaactgacaacggcaaatatggacaagttacttgccgtgcaggaagaaattgagtcgtattttgacagtgaattagccgggcagttctgctacacattcgacgactacgacacaaccatgcaagacatcgttcagaccatcgcggaagccgtgttttgtacggcataccgtaaaggtgctgatattatgctgcgattcgaccgtcctgttgcggggcctgagatggttttcacccaccgcagcaaaacgaccggtacggagaaatggacgcgcacgttcaacgattcgacaacctacgatagcctgtcgttctcgtacattgacccggatacaaacgtacaggagacgatttatatcccggaagaactcggcgcgaacaccgaggagtacgaatcgaagggtgtacgtaactatcagcaagcgtactggctggcgtggcgtcgctaccagcgcaacacgttaagtaaagttgtcgtagagttcgaagctaccgaagaaggcgctctcgctactcccggcggcgtaatcagtgtggttaaaggctcgcgtatcgcgccgcaggatggttatgttgttgccgtcaatggccttacgctgacgctgtctcagcctgttacgtttactcctggtgatgaccattccatcattcttaagaagcgcgacggctctgtgcagagtatttctgttatcaaaggaagccacgaccgcgaagtgattatgctctccgcgccggaggaggcaatctacacggggaatagtgcgctaaaaactgagttttcattcggcaacgaagcaaggcataatgctcagaagatagttgtttcttcaatcgaccccggcgacgaccgcacggtcaagattacgggctacaactatgatgacggattctataaatacgacggcgtcgcgccatacggcagcggtttctccgacggattcagcaatggttttaattaaagaggactctatatgtcaagcggatgcggtgacgttttaagcctggcggatttacaaaccgccaagaaacaccaaatttttgaagccgaggttatcaccggtaaatccggcggggttgctggtggcgccgatattgattacgcgaccaaccctgttaccgggcagacccagaagacgctccctgccgtgttgcgtgacgctggtttttctcctgtatcgtgggacttttccaccggcggtacgttaaccgctaatgaccgcgacaaagtggtgtatgaccctgtaagcaagacgtggtactcgtataccgggactctgccggttgttgtccccgcatcgtttaacccggttggtaacgctaactggaagccgcagactgacccggatttgcgcaatgatttatccagcacagacaatgcgacattaggtgatgccatggtcggcgtccgacaaccatttaccgacgctgtcggcaggacgcaacacgataaaaatagagaagtagtttccgttctggacttctatttaggtactgaccctgattacacaaacgcccttaaccgagcgcttacagctagtaacggggtgcttgtaccgcaaggggagtatagtacgtcgctactctcccacccgacatgctctctattcggaacagggggtggggttttaaaacaatcaaacgattctggaaaccacttaatctttgataaacctgcaggagggctacttagcaccctgagtattgtaggaaataaggcaacggactccacacagggtcagcaggtttccttcgccggtgggcaggacgttactattaaaggtattgattttaaaaatgcaaagggaactggattaagtttaatagcataccctagcgatgggggtccgtctggatacattgtaagcggcatacggggcgactactccgggtatgctacaaataaaaaagcggggtgcgtgctgtttgattccgcaagtaatactataatcaacgatgttatcgcccgaaactacccccaattcggggcggttgagttgaaaacagatgctaaatgtaatgttgttagtggcgtcattgggcaaagctgtcagcacgttgtttataatggcaccgagacgaccaatgcccctagcagtaatattatcagtaatgttgttgctaataacgctaagtatgccgctgtggtcaccggcaagggttcaggtaatctggtgacaaatgttgtagctgattactcctcctccgaggccacgcaagcacacggcgttacattacaaggcaactataatgccgctgataatattctaatggttgggtgcagcggaactaatagtttagggcaaacgcaaaccgcgacttctattaggtttttagacggagctagtaataactacgcatcggttttccctatgtatagtgcttccggggttgttacactagcgacagggactacccgtaactttgtggaagtaaagcaccctggacccaagaacagtcttcttagttcactatctactataaccggtgtctctagcattgatggtactaccgccagtaacgtggtacacgcccccgctataggacaatacatagggtccatgtccggtaagtttgagtggttcactaagtatatagatacttctgcattgccttttgtgacagctgataaattcagactaatttccgatggggccacatctttggctattggtggaggtacgacctctcagataaaattactcacatctgatagtacttctcgaactatttctctggttgatggtgatttacgcttagcctctgacgcatcggcgtatattcaaatagccccgacggctattacaccatccagcgcaaacaccgtcgctatcgggtcggcaagtcgcgctttgtccggcggattcactcaaacagcgtttacggttacgtctgacgagagagccaagacactacccctggaattaactgacgctatgttagacgcttgggctgaagttaatttagttcaatataagtacctggatagggttgcagagaagggggaggatgcagctaggtggcactttggagtagtagcccaacgagcaattgaggcgtttacccggcacgggttggacgcgactaagtacggtttcctgtgctacgataagtgggaagcgtctccggaaattattgatgaggaatctggggaagtattaacaaaagctacggcggcgggggagcggtatggtattcgttatgatgaggtattgatattagaggctgcgttacagcgacgtaaagcagctcagttagagaaaaggattatagcgcttgagacattagtggctaccctgacaaacagttaaataaacaaggccccaaacggggccttttctctactcttctgataacttctccagtacaaacgccagttgcgcattagcggcgtctctttgctgacgtagccgcagaacctcttcttcgagttccttgatacgtttttgcaatgctggaatcggggctatgatgttcatctggtaaatttcctcgcaagatacgttatttcttcttcacaaagttcatcaaggtcgttagatacaaatcctctggtgaatgttttgctgaactttaatccagctttatcattgtcgccagcgcacacccagtcatacggcaaaagtgacatttgctgccgtaggtctgttgatatatttgaccccagtgcgcttacagcattgaacccgcaattcatcaaggctacggctttgaatatgctttcggtaacaaataccaccccgctttccggcaaatactcaagcccccataaacacggccttgttgttctggtaaagtaccgcgcgtctttagggtttttacagttcttttcggcatgtggtttgtaatgctggtatccgcgaagcctaccgtcaaacccccacaggtaaaacgtagctactccaggggctaagactacctggagacggtcagcgtcaaacccacgcgccagcagatgagctttaagtagaaactcttcgaaatccatcatttcttacctcgtctcttcatgtaattaagcaactcttcctgtaccgatttcttctcgtcggtacgcgcggcgacaacctcgtccagagtgtctttagcaactatgtgataaaggaacaccgggcgctcgtgacccgcctgtttctggcggactgggcctatgcgctcaacaacctgcaaatagtgctcaaggttccagccttgcgagatgaacgccagatgatgacccccgtcctgtaaattcaaaccatgcccggctgacgcaggatgcacgcataaaatctcgatttccccacggttccacgcttccatctgcttgttccccctagcgcctttggcgaacgcctgtgcctgtgggaatcgcttaaggatacgctccagttcgtgtttaaactgataggctaccagcaacggcgcaccctgcaactcctcaacaatcgactcgagcgcatccagtttcgtgtcgtgcactttctcccagtctttggtcgcttcgccatccggccctgacacatacacggcaccagatgcaatctgcaagcactttgaggtcttcgccgcagcgttagccgcttcaacttccccgctctccagttctgcgaataacttctcctccatatctatgtacgcctgacgcgctttcttcggcaggtctatttccaccggtacgataacaggcgcttcacaaccaaaccactcggcagggtctatggtcaggctgatgtctttcatcttctgatgaatctcattatccgcacccggtcgtgcatgatactcgcgggccatagccgatttacctttctgtaccgagttaaaccagcggtcggtgaatgctgtgtacgaagagccgaggcgctcgccagcgtcgataaaccagttctgaccccacaagtctttgaggccgtttggtgacggtgtgcctgtcaggttgatgaaacgcttaacctttccgaacgcaaccttgctgagcgcctttgcccgcttgctaccacccgaacggctgcggaacgatttaagcttcgtgctttcatcggcaacgataaccgtaaaaggccagtcgtctttgccgtagtagtcaattagccactcgataacttcgtagttagtgcacaccacgttagcatctgactccagcgctgcgatgcggcgcttctccgaaccagttgcatctacgacacgcagacaagggaattgccatttctcttgttcagcgggccacgtaccggatgcaacacgcaacggggcgaggattaacacgcggtcatcttctgtaagctgcccgttgcgaaacaggcgattaagcacccacatagttgaggaggttttgccccctcccatgccgcaccagatattacagcgcggatgctgtagcatgaacgaagtcatgagcttctgatattcgcgcctttgaaacttactcattttgccaccagaactaactctttacgcccgaacgctgtaacattgcctgttacatcttcgataaccagtttaccgttcgactcgacgaacactgtatcaacggcaacaggacgacgtgttttaacgttgaaaatcatgtcacccggtacgatgtcacgtgctggtttacggtcatattcgtatttcatctatcaattccttatattgttggtgtagggctaactataatagttcgctattaggtcgtcaacctgtttgaacgacccgacgacaaaaacatttgcaccacgcttacgcatccgctcgtgctctcgtaactggtgcgggtcaggcttcgtgctttcgtctttcttcacctcgacgaaccagacgatgccgccagggagaattaccagcaggtcgggagcgccggaacgcccctcataagacagtttacggacgaggcccccaagggcctcgaatcgctcttttgcgtatttctgtatttttccttccggggtcatgagcgcagaacccaggttataaatgccccgcccagaatggcaacgccaacaaacttaaagaacaggccgtaacagaacatcgcagctattcccgcacctagtaacagcgcgagcagggttactattgtccaaaatacaaacattgtcataatacacacccctcacgtttcgtatgctcaatcccgcagcgcggacagattcggcagtcttcttcgtataaccagtaaattttcattccagcacccacaaataaattgcgatgaacatacctaatacggcgaccatcatgccgtattggccctcgtgacagtagacaccggcggcgaatcccgccagtaccgcgataatcagtttacttggcattctaacctccgtgattctcatgaaagccgtagcgaacaatcgcagatttccgggcacaagccgcgtcaaatatattgtcatggtggcccaggaatataagtttaccgtcaacgaatatccctgctttccatttatccgcccgtgcgttccagtgcacaccagtgaggcctgacttgttatcttttctgcgagatgcgtttcggttattatcagtacggggtactttccgaaggttgcatgcacgattatcatccaggatgtgatttatatggtctacctcatcatcaggccctaaacggtcattgttatacatctcccacgcgatgcgattagccctgtaactaacccctctgacgacgatacagatgtagcccctcttacttgggctaccggcttcgtctccggcgtttatactgtgtctcggggaatacttccatcgtatcttccccgtgtcaggttcgtagtagaaatggtcatgccaattaattaaatctctcataaatcgcccctcatcatttagcatatctgtacatttcgctaccttccgctacaagagggaagccttctgcccactcaggcaacgcgcacatcaatcgttccagttcagccacactgtattccggcgtatctggagtttcgcacaccagttcatcgtgtaccgaaagcacgatgggatacccgccatcctcaaccttaatcatcgcatatgcgagtaaatcccggcacagcgcctgaacaatgttttcgcaggctttgccgccgtgtgtgtacagggtagtccattggcgggttaactggttttcaccttgatacttgattcgcacattcgtgttcacccgtccgtcttcatctgtttcctttgtcacactaaccccgattcccggatacgagaggatacggccagacggcaactccatacacaaccaccaacccggaaccttcctaccggatgaatcaaattctacagtacgccatatgcggatagccctttccccatttctgcgcaagtgtgcccccgcccaaaattcacgaccaggattacgcacagcggctaaaattccatctttaaggtcgcgccagaacgctactgtttccgggtgtgactcgcgccacatacgcttgatagcgtcacaagtacgccatacttttttatcaagaatatatgatggcctgtcgtccttttcacctggatgcggggggcgcttggcttcctggatgcgcgcccattcatatcctctcgcggtggctgaccagatgtggtcggggaatgtaccgtccattgtttttgccatctcaataaggtcaagacctaagtttttggcgaacgtaacgaacgctccgacgccgccttcatagccgaggccaagctcgcaagccttgcctatctgtctgatttccttgaagtttttcttaatgtcatcggggtccatgccgaacatcttacccgcggttacgcagtaaatatccagtccggcgcggaacgtatcgagcgcggtttcttctccggccagccacgctaaaccacggccttcaacgttagagtaatcggcaacgacaaacttataccccgcttccgggataatgcagctacgaaccgtagatgctgttagcttggctacatcaaaacggcgatgcgctcgacccttaagtaacgctgaaatgcctttatccagttcatcatcgtgatagtaacctcgcgccaggttctgcggctggaatcctttacccgcccatcgcagagtacgtttcgctccgccgtactgcaagcaaccacgacggcggtcgtcagaagaacggcccaacagcaacgggttatatttcgttgacgcggtggacgcagcccctaggcgcatttcgataatcgtgcgagcgtcgtccggtaaatcatcatctgccaacaggtcgttaagcgtcgacttctgtgcattgtgtatgtggtgcgcgggcgcaagttcacgcagaatcggaaggaagtctttaccggtaagcgagccgccgtatttacgttgagcttcttcctgtaactgtgccttgtgcttctctacggcttcaatcgcggcttccgccagtgcgacgtcaaccttaaatccgcggtcgttgattaactggtcaagttccagtacacggtcttcgaactcggagttaccccaacgcggcagcttatggaagacttcacgcatcgcagtgatgtcgctcacggcgtacctgatgaacatcgcccactcgtcagggtgagtttctgcggtgtagcggcggattttgtagttcttcggcgtcggtttagagaaacgcttaatcagagccttgccgcgtttatctttcgcgttgtctgcagacacgcccagcacttcgcacagcgcatcaagagaacccggcagcgcgtgacggaacgcccaaatcatagtatcaatggtgttacttaccggaatatcaaagtcccagcagtgtttcatgattaggcgatcgaaaagtccaccgttgtgccacaccatcttgatgcggctgttgggcttaacaaggcggcgcagtgcgcggtgtaaatcccccggcatgtcgctgccgtcggtgcaatcccatacccgcacaggttcgtcgtcaaaagcatatgtacagataagcacttcggttgacgggtgttcggcgtaagcgtaagaaccgactttcttcaaatcggcttctgagaatgtttcaaagtctaagaacaggtaactcattatttttgacccctagtaaaaaggcccaatgaagggccttagttaaattgattcagatgttagcggcggcgacgttcgcggcgcggtgcttcatcttcttcgtcgtcttccaggtcattgacgctcgcagcgactttagaaccgccgaacgctttgccttcgccaacgtatttaatcgccagcaggttaacgccgaggactttgtatttctggctgaaccagatttcaacgcttacgttagctaagcatccgctgtaaacctgttcaccttcaatctgttcgccgtctacgttgaagtcctgctctacctgagtctcaccttttttagaggttacaatcagcggctgtttctgtgccttcgctttgaagtagaagccttccgggaagtcttcaaacggattgtcgcgctcggcaatgtctttaatcgcgcatttatccatgtgcttaccttcaccgtagttggacttcatccatttctcggcagcggctgcgcctaacgcttcttcaactacagcgtaaacggtgtcgtagagcgcgtcgatttgcgcgtggtcggacggcaggataatagtcgcgctgtactgacctttagtgattgaaccatcatcattttcacggtctttttcgcgttcgaatacgttaacccaagcagtgtttactttacgcagatttaatttcagtcccatttctcgattcctcagttttcagtttactccgggagctgcccggccagtgattagaactataatagctaactattcaggtgtcaacactttattccaaatcttcttcactaacctgattccactcaggacgtttgtcatctgccgttgcgacacatggtgcgcctggcttacgtgtaatgaagtctttcagttcatcttcaggcacaactttaaccgcttcggttggcgtcatgagcacttgcttcattagcgctatgccatacttgccagccactttctccgcgtctttccacacgcgattaccctgacgaccttcaaccagcttgtacccaggcactttcttaccggaatgcaaagcggcagccatagctttctcaaccttatcgatgtgctggcgcagcaacggcaacttctcatactcagctacgagttgttcaggcgtcagttccagcgcaaagtcgtcctccagttcttccgccagtacagaattaaccgtctttgtacgcgcagcgcattgttcagagaaccggcaccactgacaaccatctaccgatggcttgaagtccgacgctttcaggttcttcttgcctcggaaatacgcatcaagcgctaacagcgcgcgtttctgtgcgaacttagcgaacagttccagtccttcaaccgagatgtcccactctgtcgcgcccccagcgtaaggctggaagatgaccagacgaacggttgttatgttataacgtctcttgagtcgacgataaacaccgagagcgtaaagcataagctgcttgttttctttcgcttcgacgcgatgccgcccggttttcaggtcgccgataatgagcatgtgctcgtcggtgtttgccagttcctggacagcaacgaggtcagcggttccgaacgtctcaacgccttcataccccggatgcaatacctcagtaagattgacacgcatttccagcttggcgtaagtcgctacgtctataatcgctttgcaatagtcggtgtacttgcgcacctgctcaatcatgtccgccgtaatcagtaccgcgcctttcatcgggctgattagcgccttaatctgacctttgccttcatccagtacgtaagcgccgacttcacgctccaacggcaacgcagtgccgcgtatataggcgttgagatggacctcagctatggtgtgcatggcggttcctaatacagcggctttacccgacgtgttagggatatctttttcacacgccagcgacgcagcgcatgacagccactttttagcgcctgacggtgacagtaaggcgtgtacatcattattgccgcctcgttcttttagaatcattatttagcctcctccggtagttctggtaaatacatccagtgtgttatacccatctctatataccgtttcgtatataactgatttccgttttcatccagcccagcagtaatgtcgtcgaaatagtcctgtatatgcacaaaatcaattccgccttccgggaacccattatcgtcacatttacttccgtctactgagcaaactaaaacagaatcatcttttgactctggtagtgcttcgtttacgctaacccaattcataccctgttctcccactggtcaattaaatgtcgtgtcttatggtcgcagtgcatggcccacccatacatcgactcgaagacataaaagtcaggcttggcgaaagttgtgcgcttaatctgtgacacgtgacggcctatatctttaggccgtggtacttttcctaagtacgccatctcttccatctggtgcgcaccggacggagcacgcaatagccatagcgcctctgtgttatcccgcctgtcgacggctcggtagagttggtaaatcataattccgaccctcagttaaagcggcccgaaggccgcgagatagttattcttcttcgaaatacttgttcttgattgctgtcaggcgttccaggtactcaaccaggtcttcgtctttaatcgcggcaatcttcatcttcttacctgtgaactcttccagcagttcatcagaatcatcgcacgcggcatcgctaggacctccattaattgcatcgtcgatggcctgaatctggtcacgcagagacttgtaatcgacttcttctttctcttcttccggttctggcgcaggttcctctactttagctttacgcggcttgcgttttggcttctcttcctccgccggtttagtgtcaactacgtcttcaccttcaaccgggatttcttttgttgcttcttcagcgcactcagctaccgcttctttggtgtacgataccgtctctacttccagcggcgtggcaacctgaacaacttgtttcgcactgttcgcggcaatcagttcatgcgcaactacgaaacgttccagtaatactaagaatttctctaacattatttattctcctgtttatttgggttactcgccgtcgccttctgtaaggctatcgtctattaattcaaatttaccgtttgggtgttgaatagcttcttgcccgcaatggtcgcagacaacaagtttatcgaacccatcaaactcatcccccaccacgcaagaaagtacaaatttatgttttgtgcacacttcctgcgattctccgaaaattgctagaaaacctttagctatggctcccgttattgtgttcatatccgcccctctcgtttggtatgggctaactataatagcgaactattcacatgtcaatgggcttttctaaaataattaatatggtactattcacatatcgactgactaaggagtaattgacatgcaaccatctgaactaggtatccgtgtagaacaacgccgtaaagaactcggcatctcccagcgccgtttggcggccctgaccggcgtttcccagggcgcgattaaccaactggcacttggagtaactcagggcgtccgtcaggcaacgctgttcaaactggcggaagttctggaagtagacgtcaagtggctggcgttaggtgaaggggcttaaagcccctttctttttatagcaacttatcgagttcttccaaattcttaatagtgtgtcgcacgttcaggtactgaatccaggcgataaaccacgcacttacaggaaaacttataacaatagttatcgatataattaatttgaaaaggcactttataatctctgccagcgtcatgtctaaaatgtctttaaactccgcaaaaatccccgctgcatacacacaaaaagtccaccagttgttgcttacagcggaaacacatgtcaggtatgacgggcggtatcctgccttcactgctttaaacgggttatctataaaatcgtaaatattcattccaaatcctcctctgtcactgtcaacatttcattcggttcgtatattgtctttggaatcttgttatcagttattctggtgttcagcctgtaacgacctgggattatctgattgttttcgtcagtacccggaacaagatacccggcctcaaccattttcttaatcttcccgcgttctatggcttctttggagttaaacgcctttgcgttggggtcagactgcgcgagcttattcgctgcggataccgtgatgccctcgttgccgttgtaggtcccctccgccagttcaaacgccgcgagtatcgtggcctcggaactgttgacggcgttctctatggttttacgtacattttgtttaccttcgttagttaacccttcttccctctctttctcctcgtcggtcttgaatggttcgaagccccacggcatcaatacaagagccttgtgcggctcaggcaggtcgaggtttactattgtgccgtattcctctgtgctaccgaggaactcaaccgcgcggtactctttcggcggcggtgcttcacggaactgtacagactccagtaccatgccaaccgtcttctgttgcggaccgtgcttaaatttagagtggtatacgtttatctgacggtcggtagcgcgttcgattgtcagttccacgtcgacacccgcatacaatgctccactgccgcgggctttctttccgcccttcggagtatggtgaacgacaccgacagcggctttagttgcatcgcgcacttctttcaggatggcgataactttacccataccgattgccgttgatgaactgttctcgtcgaacttatcaatcgtcagggccagcgtctggttaagggtgtcgaaggcaaccatgccaataggttcatcccctgcggtttcgcgcatcctgcggattagagctggaatttttttatcaccatgcgtagcgagtatttcgcccatatcgatgacatgtacataatctttaccttcctcgccatatttagccgcgagtgcatcaatacgtgttcgtgtagctgcaccaccctcgccgtcaatatagaaatggtggcaacgttgggtgtcagcccccgcaaaccggtacccggcggcgctcaggtacatcatccccagcgtatagaacgatttgtacgtgccagattccccgacgatatcccagatacaatccgacggcatgtacccctcaacgacgaaatcagcctttaccggctccggtaactcgtcctcctctgagtcctcgtcgtcttccaggtcgtcgaggctgcatgagacagattcacgcgccccccaaccgatggcctctgcgacttcactgaacggcagcccggtcgcatcgcacgcgtacttccacacctctttcggtgacaggccttctgtcgccgtaatgtctgtgtcgtgaatcatggttacgtttggcgcttcatacccctcgcgcgggaagcacagcaggaagtcgtccgggcgcggtgtcgggtcgctgtagttttcggcatgttccggtgtggctggcatcttaaggccgcgcggcgtcatgacgccgccgtactcaaacgccagtgcttcaaacgcgtctgtaaacgcggtgcgcagttcttccggtatctggtaatccgatgcgctgctaacgtcaacggctgggacgccttccagtaactcgttcgggtcgatcaggtcgttgcggcgcgaccagataacggtagcgccgaccggcggcaggtacatcggctgcgacagagtgaacccgctgcggtccgcacccatgcctttgaagaagtgctccagcaacccatgacgaacacggatgatatcaccaccctcaactgggcgggccagcggcatgacgacgcgaaagcgaggcgactcatcggtatgtgatgccgtggtgtagagacacatcgcccggcggctgcgcttaaccaggcgcaccgcttcctggtactcttccggtgttgtgctgtcgaaatccagataggccagcgacgatttgcttacagacgcatcgcagcggtagaaaaaacctttacgcgcttgcttaaagtctccagtttccgggtcttttacggtgctgtgcgttgagtcgcacgcggcggtgatataaccgggcgcggtcttagggttaatcccgtcgcgaacggcatcgagcggctggattaactctttcaggtcgtccagtgttgccgtgtgtgcggttctgacatttatatcctttttccccgcccgcgcgttgcggcgtgaccacgagtaggataaaattacatcggacatgttgtatttccttcagcaagtaatttagcctcggcgctctaacgtcggggctttcttttattccaggtcttctacagtagcggtcattccgcgaacttcagcaactgcgctatatttcccaccaacatttttcacgacaccagatttaaccagtaccttcaacgacccttcaataatggcggaactatagtacttaaaataactacggcgcaagtccataacgctgcacgacccttttttacgtgttaatgaaacgactgccgtaaatacgcgtgactggaactcgctcattttacattctccttaatccacgcttccactttctcccggtcaaacgtacctggctgacggcggcccataatgcggatacaacaatccgggaacttcccactctttaaccagttattcagcgtgcgacgggtaaccccgatacgctcagctacctcattctgtgtcattctcaaaccctcattatcagttaacgaaactgagtatacattgcgaataatgggaaatcaaacataatcgcacctattgacattatgaaaatcttcgtttaaggtgcttttatatcttagttactttgattcttgttcaccttgtaatacccgcttgaaacgcagcggcgcaccagcgccagcgaagtgttaagcggcagattactgaacatatgaattatcgtaactttccttcctaagtatctccggttgccctgggcaagctctattctcatcgacggcatatctcttaagtatctgataattaaaagtttctatagttgccgtgagcaaggtagagagtacttcactccgctggggtgggctaacgcccacccactgcgttgcgtactcttttaagaaacgaaagaatcacaacggcaacgtaactattctcttgcacaccccaacataataggatactattcacttatcgaatcgagacagaggagtgagggttatgcttaagaagggtcagttggtccgtagtaaaaagtcgggatgtttgtactccatattttccaccaacaacagaggcagtgccaccatttgtaaacttcgcaatgtatttactgacggccatgcaactgtaagcgcggaatatttaacactcatcggtaacaattttaaattcaaaggggtgaagtgatgcaaatcataattacagataacaccgttatctacgaagaagatggtgatactctcgagaaaataggcgtaaatgtgggtgatgttttcaatgtactggattcctgtgaggatggctggtggattaagacaggaagatacacaatcccggtaactaaggcagaagcgaaggtatacacaacggcatctaatcatgatgctcgtgccgacgactctgagggaggttgccgtgaataatattttaattgcgggggttggtatgagtccgtataacgaattccgcttacgccgtctgattggcggtctgcgcgccgccgagtttggtgttgaatgctgggaaaaggcgaagtacaccccgtggaagtcgtggcatttggctcatgctaaggcggtagcacagtaccgtgagtacaagttaaacagttttcttaagcaccacggggttgagttatgagagaagcatttgaacgtcgggccgttgcagatggtctgcctgtcaacaagggctcgcggaacgagtaccttagcgctaagacgcgtctcgcgtggcggatgtggaaagctggtgtgcagtatgcgatgaatacgaggtgagatatgggcgagtggattaagtgtagcgagcggatgccagaaaagaaccagagcgtacttatttcggtgaatttcgatagctctctggttgagccgctaatatgctccgcacgctataccggaagcacatttcggcgaggagatgcaacggttaagccgggtaatggtgttgagcaagcaactcactggatgccgttacctgagcctccggaagggtgatgttcaatagtttgggattttactgagtgacttacgctgctacacagcagcgtacaactttaacttagtgtcgtcaaaaagcgacactttcaccaaacgcaacaatcgaagcgactattgcaggagatgcaacaatgaaactgaatgacatcgtaacctggaccagtagaaacggagaaaagcgattcgggcttattgttgcgtcagacggcagcaagtaccgtgttatgcgatggcgtcagtgggcacgacgcccgaggtactactggattcgtagcgaacgattatctttaaaacaccaataaaatttacttgcacactaagatagaatagactactattcatttacacaaacgagaggagagacagaagatgagtaacaaaaacgaagtattcgagtacctgattgaccagttacggcagcacgtaaatagccacccatacaagcaacagtgcgaagacctggcacatgaggtgctgtcacttaagaatcagttacgtgatgcgtcggcgctggtggctgagttgcagagcgagttacagcatcaaattgacatggcggcgggtgtgcatagatggtctaccgcatatttcgacgagaaaggtaaagtcttcaaggtcgagagtggggttaagacagagcaatccggttgccaaataggtgggcatgaatgggtggcgacactgcaagatgatttccgtacatgcagcaaatgccatcgggaagagctgatatgaccagcatcttatttatctgggtactgtccgcaggccagatgcaactagcggcatcagaaacgttttactcaatggaggcgtgccagtaggctgcccgcgctgcagaggacgcgcactttctgtttcagggcgacaagctcaacgattcagaggtacgcgctatctgctcacctaagcgacttggtaaacaggagaagtgattatggtgcagagatatacctacgaccagatattcgggtttactcctgatgttgagggcgtgttagtgctttacgaagattacgcgaaacttgaagctgagttacagaaatacaaggaccagtaccctgattacgtcgagtgcgcgaactgtgggtcggttacacatgtggagggggtggagtgatgtcgttagcaactgacatcctgaaacgaagcggcattgcgccgctgtcaccgagagcgaagacacgtatacacaagcgtcgccgtaacgtgctgtacccagagatacaagaacggcgtaaagctatccgcgcctgtggattccagaacggaaaggccgttaacctcggtgagtttaaaacacaggaacgcgcagctatcgctaatcggttatttaattactggaaatcgctgggatacgatgatattccatcgaaaccgcagagacgacaatacatctggcgtcataaataaaccgttattaagataattcctaaccgtgctatcctccagttactgcatacttaatacgcacctggaggattcatcttggataaatttactgaaacagtgacggggtggcttctcgctgccgcactggtcggtggattggtcggactaagacaacataaaaagtctatatccgggccgattgacggactggtatttcttctcaccggcttcgcgtgcgccattttcggcgcacctcttgccgctcaatggtttggtattactggcgagcgcgagatagctggcctcggattcatcattgctattctctggatgccaatttattcccgtctctctggcattgtcgccggagaatacatcgcacgtcgcggaggtggtaatgaatgagttattctggtttggtggtatgctttcaatgggcgcttcgtccctgttcaacgtgtataacggacacgtgggcgacgggctgttcgggcgtgtgctttatattctgactgctattgtctgcgccgccggatgtatccacctgttacagggcagcatgtcaccgacgctgcctgagacattaatcacattagttgcgctgcgtcagattcgtcaggcgtggctgtcgtacggaggacataagcgtgtctcgaaacattagcaacaatggcatcaaattcaccgccgcgttcgaggggttccgcggaactgcgtatcgtgctacgccaaatgagaagtacctgactattgggtacggtcattatgggccagacgtaacgccaggcaagaccatcaccccgggacaaggcctcctgttactgaatcgtgatatggccaaggcagtagcggcggttgatgctgcagcgcaccattcattgacacaggcacagttcgacgcagtgtgcgacctggtgtataacgcgggtgccggtgtgattgcggctactactggcacaggtaaggcactgcgttctggtgatattgcaacgctgcgggctaagctggcgctgttcatcaaccagaacggcaaaccgttactaggcctgcgtcgccgtaccgccggtcgtctggcgctgttcgacggtaaaccgtggcaggaggctgaggctatcgggcgcgcggtgaaaggttgacacataagactaatccgacgatacttaaatcacctcctgctccatccctctgctctccagttttatcccggccctgacccagccgggatttttttttatctattttctgtgatgactagttgactattatcctcgaccctattatatttacttcatcgacaacgagaacggagtagagaagatgagtaacttccataatgaacatgtgatgcagttctatcgcaataatctgaaaactaaaggggtttttgggaaatgaaaatcacagataccgaagcattcgaagacgcgcaactgatggcacgcatcgccgttggcaaccttagcggtaatatcccggccgacgcgttctgggccgccgcgatgcaggcactgaaagcagcttatgcaggagagaagaaatgagcgaacaaggtcaagtaagccaaccattacgagtaggccataaagtcagtcacaccccgttcccgacacgcgaggaactgatgaaacgtaacagtttcccggggccggacaagaacaagtatctcaatcgcatgtggggagagcgtaaagaatgaccgaccgtgaatacgaaaagatgatggtggaggctgttaacggcggcgtagacatcggccatgtgatgcacgtcctgaatactaaaatcgcggtagccgagcaaatggtggagtcgctttatgagacacgccgtgaactgattaaccgcttcaaccttaacaaggcctcgggtgatgggtatgaaagcgcctgaaccggtagttattgatggcgtcctgtggaaaccatactcggttaaccacatcgacgccgacgggaagaagtttagcttctacattttttgcaattagccgtgagcacgccgcttgtgtggttgactatatacgggaaacggcgtggcttggtgatgagatagtggggtgagagtatgagtctagaggtggttattggccttgtagcagcaggttattttatcggcgtattgattgggtttatgtggggtagagacagtgttcagtgacatcaacgcagcaatcgaagaggcaatctggcgccgatacaacggagagcagcagcggcacttctgcctggtgcaacgcggcaacatggtcgccgtagtgcaggaccgcgataacaaatatccgaatgcgatgtggacgacgaggaatttcttatgatgattaccagcattcctaaccttattaaagaatttggcacgatggcggagacgtgccgacaaacaggcctcaacgaaatgacgattgcgaagtacagcaaagacgtgaaatgcgatcgccatgtaatttataataaccgccttatgacgcacgttaagacaagcccggtgctattcacacgccgcggtatcactaaaactgaacagcgcattgctaaaggggagagcggggaatgattgagattttgagggctacaaatgctgctggcgacctggtgttttggctggcctttctcggcgtactgataaaacaaccgactttgtttaacagtattccttgctatctgtggtggcctatgtttttaggcatgggtgtatcaggagtagctggcgtccttttgtggtttttcaaatgagactgctaatcatccctaacgcctgggctattgccgtagctaacgaccattacggcggcgacggtaaaagagcaccacgacacggcctatataactgatacaagccctctacggagggcttttctgtacatcccgcccaatccccttatataatccctttagacgcgtagggcgcgtctggtgcgctctgatggtcagacgcatatgcaaggggattctatgaagctgaaacttaagcagccatcaccagaggtggtgcaagctgcacatgaagaagccgttagcgcaaaccgtcgccgtaaacgaccgcgcggcaaacagagcctttatcaatcatcccgtaattctgcggcattgtgggacccggactattgcgatgcactaatcgagttcttcgaccgcacgtcgtgggagcttgtgcctacgtctaagggtgacgaacgcccgctgattcaggataaaccaccgtcactggcccgcttcgccttacacatcggagtcactatcccgattattaagctttggctgcgtgagattcccgcatttgcagaagcctgggagacagcacaggcgctggaagaggcatacttcactgaaacgggggccgcgggcatctctgctacgtttgctgccgcgaaactgggcctgaataaaacagttgtcgccgaagaagtacgcgacgagccaatcagcgaagtaacaattaaggtggtgtccggtgaacgttaatatcacggcaacggagccgcaaggcgcgtttctcggtatgcattgcaagtttccggcattcgtagctggcttcggtacgggtaaatccgaagttatgtgcaactctgcactactcgacagcatggaaggtggtagcgattctatcatcgccatgtatgagccgacttatgacctggtgcgcctcatccttgcaccgcgtatggaagaaaagctcaccgactggggtatccggtacaaatacaacaagtctgacaacataatctatacgtcttccggacaatttggggattttgttctgcgtacacttgataatccagcacgaatcgttggctacgaatcgtttcgtgcgaaaatcgacgagttggacacccttaacatggagcacgccgagcacgcgtggaacaaagtcatcgcccgtaaccgccagttgccgcggacatataaacctattacaccgaaacctgctaataccgtttccgtgttcactaccccggaaggattccgtttcgtacatgaccgctgggtagtcaaaaagaatccaggctacgagatgattcaggcgtccaccctgtctaacccgttcctgccagaagattatgtgcagtcgttacgcgacacatacccaggtcagttgattgacgcctacatcaacggcgagttcgtcaacctgacggcggggactgtctattacgcctatgaccgcaggaaaaacagcagccgcgaaacaataaaaccaggcgagactctgtatatcgggcaggactttaacgtaggccacatggctagtacagtttacgtgcaacgtggcaaagtctggcatgcagtcgccgagttggtggatatgttcgatacgcccgatgtggtgagagccgtaacagagcgctggaaaagtaagggccactatatcgttatgtacccagacgcaagcggtaaaaaccgtaaaagtaacaacgccagcacatctgatattgcccagttacagcaggccggcttcgaagtgcgcgctaaatcgacaaacccaccggttaaagaccgcgtagcggcgatgaataaggcgcttgaatctggtatggtcatgattaatgaacaggcttgccctgttaccgcacgatgcctggagcaacaggcttacgacaagaacggcgaaccggataaatcaggcggtgtggaccaccagaatgatggaaccacataccctatcgcgtatgaaatgccgattcgcaaaccagttattaacgtcccggtgactttcgcactttaagaggattattcaatgttaactatgaacggtcagaatcagggtgttaagacaaaacaccgggaatggctgcatcacttcgataaatggcagaaggtacgccacgctcttgaaggcgaccttatccgctatctgcgcaacgtcgggaagaacgagcctgaccagacctacgcagcacagcgacaggaagaatacgagaacggcgctatctgctacaatttcaccaaacgcacgctggtggggatgacggggtcagtgatgcgcaaagaccctgagcagattatcccgcctgaacttgagtacctgttgcgcaatgctgatggttccggtgtcggcctgtggcagcacgcgcaggatacgctaatggagattgactcgatgggccgtggcgggttgctggtggacgccccggagacagccgcggcaacggcggcagaacagaacgcgggattattaaacccggtcatcgctttctataccgcagagaacatcatcaactggcgactaactcgcgttggttccgttaaccgcgtgacgatggtcgtgctgcgcgaggtgtgggaatactcagaaccgggttcagagttcgaaacaaagttcggtgagcagtatcgcgttctcgatttgattgacgggcgctaccgccagcgcatttaccgcttcgacgccgaaggtggcacacaggatgaagtaatagagatattcccggaacttggcgaacagttgcgcggcaaaatcccgttcacgttcattggggcgggcaacaatgatgcaaccattgacgatgcgcctttgctgccgttagccgagcttaatattggacatttccgcaacagcgcagacaatgaggaatccagcttcgttgtagggcagcccacgttgttcatcgccccaggcgagaacatgagcatggaacaatggaaagaagccaaccctcacggcgtgcgcatggggtcgcgttctggccataacatcggtcacggcggaaatgcgtttctggttcaggcgggagagaacaacctcgccaagcagaacatgctggataaagagaatcaggccatccagattggggcgcagcttatcactccgacgcagcaaatcaccgcagaatcggcccgcctgcaacgtggtgcggatacgtcagtcatggcgacaattgcgcgtaatgtaagcatggcgtacaccgatgcgttgcgctgggttgctgcgatgcttggattgcgtgaagacaccgagattgagttcaaactgaatatggagttcttcctgcaaccgatgaccgctcaggaccgctctcagtggatggcggacattaacgcgggcctgttaccagctactgcttactacgcggcattgcgtaaggctggtgtaaccgactggacggacgaggacattcagaacgctatcgaggatgcgccgctgccgattggcggggctactccggtagagggagagattccgcagtcggcgcagcaacaggacactgctcagcggtaagttcgcctatagccccgaaaggggctttcatatagtatgctattaactttagcgccacagggtttatctatgagcttacttacatctctaatcagccaccagatatggctgcaacgcaccgcatccggtgaagtgaaagacctcacgccgttcattcaggagataagggatgaaatcaaacggcaggtgctgttattcggtgacgacgggcgaagcactgcccgactgaataaattgttacgcgaccttgaagaagcactggtggggcttacgggcgactggcagacaaagctgacagaagaccttaaggaactggcggcgtatgaggctgagtggaacgtaaagacactgaccgccaacgtagacgcggaatttgttacgcctaccgctgagcaggtatgggccgctgccgagtttcaaccattatcattgagcgacaagcccgttgatttcaccaagctgatgtctggatggggtgaaacggaagtagcacgtcttgtaactggagttaagatgggctttgtgcaaggtcaaaccacacggcagattgttaagaatgttgttggcgctggtggactagccgacatctcagaacgtaacgcgactacggtaatccgcaccgcgctgtcccacgtatccaacgaggcccgtaacgagacgtaccgccagaacgacgacatcatcgagaaatatgagtgggtgtcaactttggacagccgtaccagcacgatttgcagggccagagacggaatgacgtgggaaatcggtaaaggtccgatgccgccagcccatccgaattgtcgaagcaccacggccccggtaatcagttcagagttcgacttcctcgataaaggcgcaaaacgcgcggctaaaggcgcggaaggtggcactcaggtaagcgcagacaccacttactacgagttccttaaacaacaaccggcgtggtttcaggaccaggcgctcggcccggtgcgaggtaagattttccgtaacagcggtatatcgccggaagagtttcgcgtaatatctgtagatggtttcgggaatccgctcacgcttaagcagatggcggaactcgataaacgtgttgctgattatctgaaaggggaataatgatgggctttttcaaagtaactgacgtaccgtctcgtcgcgtagtccagtacgcccgcgtgtctggctctggcgagaacgtggtatttattgaggacgaaagtgtactcggtacaccggtagatgatatgccgtttgcagataaaaccggtattgcgttgcccgccgctggtatgctttatgaaattccgtatctggcggacgctggcgacgtgtatttctctgcgcaaccgcaggacgctgaactggcgggcggcagcgcaaccatcactgtcgaggttaaggcaggcaaagcgccgtattctctgacctggtacaaagacggtaaggaagtggtgaatgcgcctgaggaggctctgtctctgacggttaatgcggtcggcgaatacttcgttaaagttactgatgccgatggggtagaggccgtcagtaaagcggcgaaggttactaagccggaatgataaaaagccccgctatggggctttatttttatatgaacatcgcggtgatagccgcagccgatacccacaaaacaaaataaaacatcacactatttgtcatttgcatttctcgtcgtatgtttgttgtaactgcgacagacgattaccggctgtcatctcgtccatagaaggcccggcgcccgtgtccataaagaacagcggaacaatcaggaatgcgcctgtaacaccgagtacaacgttagtacctatttgcttattaacacggtgcgtagcgttggcttgagcttgttttgtcgtggcgattctcgatagtaactgattacatgttgccgttgtatcccccgcctgataaacctgtaaagccgggtctggcaacgaccttacgcaaccactcaaacaaacggctacaacacctgctactgctaatttaatatatttcatagttcacaccattacccgtgtcaatgtcaccaataccactacaagcccaaagaaacatcaccgcatcaactgcaattactactgaaataacgactaacatgacggcctccccggttcgatagaatgaatagtaccctattatattggggtgcgcaaactatttatttacgtattccagttattccaccgaattgtaaatgttggaataaactattcgaatagttgacttttcactaaaaatgtgataagctccacctgagcttgtgaagtatgaacaagcgaccgcggcgcgggcaggtaacggagcgggacgtaagtcctgagtgtagttacgctgacgcgttcggaagggccatactctattgcttgtgtaaaaagtaactggtttactgagattacgccgtttctatgtttaaatgataaggactagcgccctgctttaaggcagggctttacttatcgagaaaggggaaacatgaatcttaaagcaaccgtcgtagcaggagcatgtttcatcatcctggcttacacacacggcatttatcagtaccgcagcggctggcacgaaggccgcgctaatctcgtttcgcagcaacagcaaaaagcacaggctgagttagctaagaaaacacaacggcagcagcaggacgaatcaaaggccgccgccgccgacaacgaaggcaagacgaaatcagaggtgattacccgtgaagtcgttaaatacattaaaacgccaggtcgcagcgtgtgcactttcgacgatgctcgcgtcctgctcaagtcccacgccgtcgcaaacgctaattccattaccggatacgacgatgatgcagcctccgtgcaaactggcagcgccaagtagcgacgctgacgaggatttagctatcgacgttcagaacgctgaatgcgtacggcagctgcggctgaaagtgttcatgttgcaggattacgtgaggaatattctggaatagttgccttgcatgttggaataatttattcttgacatgtaaatccgggtggcccgggttccaacgtccaggggacatactgactatgaatcgttttttacgttatccgttccaggaagaagctggggtagaagataaagctggtggcggtgacgcgccgaaaatgttcaccgctgaagaagttcaggcgctgattgagaaagaagttgccgggcttaaggctaatcaggaagcattgttggcggagaagaaagaagccgctcgcaaagcaaaagaggccgaagaagaacggcagcgcgcgcaccaggaggcgttaaaagccgctggtaagatggatgagttcgaaaagacgattcgtagccagtatgacccggtgttagccgagaaagacggtcgcatctccagaatggcagagcgtatcctcggcagcgaacgtaaagcggtgctaggctctttcgcgggtgactttattaccccagaagcagtggacattcttgcgccgttcgttaagactgagttcgaaggcgatgatgtggttactaagtttgttggtgcagacggtaacgtaatcacgactgacccggaacagttccgcaaatacctgcgcgaacacaaggcgttttcgcatttgatcaaagcaaatgcagcttccggcggcggggcttccggtagcaaaggcggcggggccgcaccagcgtttaaagacatgagtgaagcagagcgtttagccctgtataaatcgaaccctgccgaatttgaacggcaacttaaagccctgaggaaataataatggcaattaccactatcggcgatatcgtaactggcaacatcccggtcctggcgtcttatatgaccgaggacccggtagaaaaaaccgcgttcttccagtctggtattctcaccccgaccccatacgccgccgagattgcccgcggcccgtccaacgtcgctaatattcctttctggaaagcgattgatacctctatcgagccgaactactcgaacgacgtatacccggacatcgccaccccgcgtaacgtgcagaccggcgagatgatggcgcgcgttgcgtacctgaacgaaggtttcggtcaggcggatttgaccgttgaactgaccagccagaacccgctgcaatccgtagcgtcacgtctggataacttctggcagcgtcaggcacaacgccgtctgattgctaccgcgctcgggctgtacaatgacaacgtagctgctaccgatgcttaccacgagcggaatgacatggtaatcgacgtgtctgctactctgggcttcgatgcgggcgcgttcatcgacgctacccagactatgggcgatgctctgatgggcaacggcggtgaagtgctgggggctatcgcgatgcatagcttcgtttatgcgcaggcacgtaagcagcagcttatcgacttcatccgtgacgcggacaacaacaccatgttcgccacctaccagggctaccgcgtgattgttgacgacagcatgaccgtagtcggcactggcccgaccagtaagttcatctccatcatcttcggcaacggcgctatcggttacggtgaaggttctccgtccaacccgctggaatacgagcgcgaagcgtcccgcggcaacggcggcggcgttgaaaccctgtggacccgtaagacctggttgctacatccgtttggttacagcttcaccagtgcagtaatcactggcaacggcaccgagactaccccgcgctctgcttcctggcaggacctggcgaacgcctccaactggaaccgtgtggttgaccgcaagcacgtaccgattgccttcctggtaactggtgtcggtgcttaaggttaagctataatcgagagggacttcggtccctattttcatttactaagaggtaaattatggctaagaccggaaaaggcttaccgcgcagccttcagaatgtagacttcagcgtcattgatatcccccgtcgctcctgctactacccgcaaagttggtggggttaaaaaggcggcccaggtcggcttccctgtggccattaccgccgccgccggggtgcagtccgccgcggcaccgactaaggaagagttcaacgtgcttgtggcggagtacgacaaactgcgaaacgatgttatcgcgctgcgcaataccgtaggaactctagtgaccgcgcttaaaaacgcaggaactgtaagctaaaggagcttaaaaatggttgatgtaatcaaacgtcgcattaccggtgtttcagccgataccgtaggcgctaaaatcgatatggcaaatatctcgccagcgtctttttctgccgcgcttgcggctaccaccgcagttacggtggggcagactatgactcttaccgtagtggtaactggcggtctgaagccgtattcctaccagtggtacaaagataacaacgccatcgacggagccaccgcagctacctatgcgaaggcgtccactactaccgcagattcaggcacgtataaagtggttgttcacgatgtgtatggtaatattatctccagcagcaccgtagcaactgtgtcttaatacaacggcccttcggggccgtaataaggaaaggtcatggcagataattacgtaatccgcgaaaagtatacccacgttgatatcgttgacggacaggtgatgcctgttcgcggtgtggtagaagcggatgaactggttgcaacccaaccagacaatgaagaagcgcacaacaacggcggtggtactaagcgtcgtcgccgtaagtcagaggaataatttatgccgctaatcgtggaaactggggtgatcgtcccaaatgccgacagttacattagtctggctgacgcccgcgcgttagcggctaattatggccttgagctgccggaagacgataccgcagcagaggtggccttacgcaacggtgctacttatgtagggcttgcagaaccgcagatgtgcggtcgtcgagtatccgccgaacagtctcttgcatacccccgcaccggcgttacgttaaacgggttcccggtggtcaacaacgccattccgaaacaggtgattcttgcgcaggtaatcgctgccgctacatatggcgagggcaccgaagtccgggctaactcagacggtcgcgccgtgcagactgagcgtgtcgagggtgcggtaacagtgacctacttcaacaatggcaacagtggcgctacgaccgcgattaccgctgctgacgacgctttacgcccgttattgtgtggcggtcttaacaatggtttctcgtttaacgtgtaccggggttaaaaatggcgaagactaaatcagagatattcacgctaatcggttccgagctaccggacaacacgaccggacttattacgcctgcgaagttgcgcggggtattaacccagatggctgactcacctatttacgccactccgggtgttaaagaggttgaagttctccgcgctgcgtcgacagtagcgcaagcgcctaccgcagtagatacggcgttgcaggtatcgttcggctctgctcagggtagtgcatctgacccggtaatgattaatgctgcggggctggttacattcaacaccgcgggtaactatgccgttcgcatcaagttacaggccggtcgctccggcgctagcggaacgtctatcctgttgtcgcgtatcctcattaacggcgctcagtacggctcaccagcagctacgaaacttgttagctcggaaaccaccatccctattgaatcccgtgtagtgattaacccaaccgccgggcaaacattcgccgttcagattatgcgagatagcgccgggactaacttcggaggcgtatacccgcaggtggctactgtaactgcatggggcacggcaccgtccgcgctactggttatttcgagactggaggctgcctgatgagcactgctttcagtaaacgtatgcaaggcgtgggtacacgcctgctaaccaaattcggcagcacggtatctttggttcgcgctggctcgaaagtgtgggacgaagttctcggtgagtacatctggtccgccgatgaagttctgccgttgaaagccgtgcctgttccggttaacgcaggtttggttaacggcacaaccattcaggccggagacatgattgtcaaagccgattgcagcgtcgttccgaagatggaggacaaggtgcaattcggcggcgagcaatggtccgtcgtagccattgagaagaaggtggttaacgatgatgttgtggcctactttattcaggtgagaaaatgagtttcgcgctggacgtctctaagttcgtggaaaaggcgaagaagaaccctgagaaggtgatgcgtcaggtgtctatcaagctgttttccgctattataaaggcgagtccggtagatactggtcggtttcgcatgaactggatggcatctggcggtactcctgcttccgggattacggatgctacggataaatcaggaaacacagcaaccggaaacgctacaagtttcgtgctgaaagccaccgactggcatgagttcacgctgacaaataacctgccgtatgcacaacggctggagtatggctggtcgcaacaggccccgcaaggattcgtcaggactaacgtgtcccgcttccagcaactcattaacgaagaagctagcaaggtgagatgatgggctactttgaggacttaacaaaagcgtttgatgtgccgctggtagccttcggaaccaccaacggaatcaaggtagcgcttgaaaacatcgacgcgccgacgtcaacagatacgccgtatctggcaagttacatgttgctggcggataccgagcaggctgatttattcttcacggaacaacgcgccggtgtctatcagatagacattaactacgcatcggtgaaaggtagcgcgccaatcaataaaatggcagacttacttaacacggcgtttaaatcaggtaaggcattttcgcgtaacgacatctgcgccgaggttcaatcggttagcctggggcagctgattgtagaaaacggatgggccaaacgaccattgtcaattaactttattgcattcaccaagaggctgtgaatatggctacaactccttttaagggcgcgaataccgcgcaattctatgtggcggaaactacccctggcgtaacaccgactaacccggtatggtcgccgttgcgtaacacgggcggcgttcccgctgtaacccgcgatgcactgacttccaacgaactggacggcagccgtgaaactacatccatccgaaccggtaacaagcaggttagcggggagtatgccatcgaacttagctctcgtagccaggatgatttccttgcgggagcgatgacttctacgtggaaagctggggtagagattactggcgccgaaattacggtcgccccagcaggtaaaacattcacccgcgctgctggtaacttcattactgacggtgtagaagttggcgaccttattgcgttcaccgacttaaccggcgacaacgcaaaaccgtttatcgtgaccgcggtttccgctctggtagttacgggcgcaggtattcagcacacgctgacagcagagacagtaaccactgacgcaaaaactggcgacaagctggaaaccggtaacgcgtgtaagacgttctccatcctgacgtggttcaagggccagtgtggtaacctggacgcgtacatgctgaccaaaggtgtggaaatctctggctttaccgtagagcaggcggttaacgccatggtcaccggcagcttcccgttcatcggcctgagtcaggagattcttaccgcgccgccgtctggctctgatttctctcaggttacgttcaccgatgagcc

SEQ ID NO: 2 - protein, 162 aa, synthetic construct
  REGION 1..162: note = synthetic_EC340
VSRNISNNGIKFTAAFEGFRGTAYRATPNEKYLTIGYGHYGPDVTPGKTITPGQGLLLLNRDMAKAVAAVDAAAHHSLTQAQFDAVCDLVYNAGAGVIAATTGTGKALRSGDIATLRAKLALFINQNGKPLLGLRRRTAGRLALFDGKPWQEAEAIGRAVKG

SEQ ID NO: 3 - DNA, 489 bp, synthetic construct
  misc_feature 1..489: note = synthetic_gene encoding EC340
  source 1..489: mol_type = other DNA
gtgtctcgaaacattagcaacaatggcatcaaattcaccgccgcgttcgaggggttccgcggaactgcgtatcgtgctacgccaaatgagaagtacctgactattgggtacggtcattatgggccagacgtaacgccaggcaagaccatcaccccgggacaaggcctcctgttactgaatcgtgatatggccaaggcagtagcggcggttgatgctgcagcgcaccattcattgacacaggcacagttcgacgcagtgtgcgacctggtgtataacgcgggtgccggtgtgattgcggctactactggcacaggtaaggcactgcgttctggtgatattgcaacgctgcgggctaagctggcgctgttcatcaaccagaacggcaaaccgttactaggcctgcgtcgccgtaccgccggtcgtctggcgctgttcgacggtaaaccgtggcaggaggctgaggctatcgggcgcgcggtgaaaggttga

SEQ ID NO: 4 - DNA, 35 bp, synthetic construct
  misc_feature 1..35: note = synthetic_primer1
  source 1..35: mol_type = other DNA
aaggatccgtgtctcgaaacattagcaacaatggc

SEQ ID NO: 5 - DNA, 25 bp, synthetic construct
  misc_feature 1..25: note = synthetic_primer2
  source 1..25: mol_type = other DNA
aactcgagacctttcaccgcgcgcc

SEQ ID NO: 6 - protein, 162 aa, synthetic construct
  REGION 1..162: note = synthetic_mtEC340
VSRNISNNGIKFTAAFEGFRGTAYRATPNEKYLTIGYGSYGPHVEPGKTITPGQGLLLLNRDMAKAVAAVDAVAHHSLTQSQFDAVCDLVYNAGAGVIAAATGTGKALRSGDVATLRAKLALFINQNGKPLLGLRRRTAGRLALFDGKPWQEAEAIGRAVKG

SEQ ID NO: 7 - protein, 171 aa, synthetic construct
  REGION 1..171: note = synthetic_Met+mtEC340+His tag
MVSRNISNNGIKFTAAFEGFRGTAYRATPNEKYLTIGYGSYGPHVEPGKTITPGQGLLLLNRDMAKAVAAVDAVAHHSLTQSQFDAVCDLVYNAGAGVIAAATGTGKALRSGDVATLRAKLALFINQNGKPLLGLRRRTAGRLALFDGKPWQEAEAIGRAVKGLEHHHHHH

SEQ ID NO: 8 - protein, 37 aa, synthetic construct
  REGION 1..37: note = synthetic_Cecropin A
KWKLFKKIEKVGQNIRDGIIKAGPAVAVVGQATQIAK

SEQ ID NO: 9 - protein, 38 aa, synthetic construct
  REGION 1..38: note = synthetic_Met+Cecropin A
MKWKLFKKIEKVGQNIRDGIIKAGPAVAVVGQATQIAK

SEQ ID NO: 10 - protein, 215 aa, synthetic construct
  REGION 1..215: note = synthetic_Met+Cecropin A+GGGGS3 linker+mtEC340
MKWKLFKKIEKVGQNIRDGIIKAGPAVAVVGQATQIAKGGGGSGGGGSGGGGSVSRNISNNGIKFTAAFEGFRGTAYRATPNEKYLTIGYGSYGPHVEPGKTITPGQGLLLLNRDMAKAVAAVDAVAHHSLTQSQFDAVCDLVYNAGAGVIAAATGTGKALRSGDVATLRAKLALFINQNGKPLLGLRRRTAGRLALFDGKPWQEAEAIGRAVKG

SEQ ID NO: 11 - protein, 223 aa, synthetic construct
  REGION 1..223: note = synthetic_Met+Cecropin A+GGGGS3 linker+mtEC340+His tag
MKWKLFKKIEKVGQNIRDGIIKAGPAVAVVGQATQIAKGGGGSGGGGSGGGGSVSRNISNNGIKFTAAFEGFRGTAYRATPNEKYLTIGYGSYGPHVEPGKTITPGQGLLLLNRDMAKAVAAVDAVAHHSLTQSQFDAVCDLVYNAGAGVIAAATGTGKALRSGDVATLRAKLALFINQNGKPLLGLRRRTAGRLALFDGKPWQEAEAIGRAVKGLEHHHHHH

SEQ ID NO: 12 - DNA, 516 bp, synthetic construct
  misc_feature 1..516: note = synthetic_gene encoding mtEC340
  source 1..516: mol_type = other DNA
atggttagccgtaacatctcgaataacggcattaaatttacggctgcatttgagggctttcgcgggaccgcctaccgtgcaaccccaaatgaaaaatatcttaccattgggtatggcagctatggaccgcacgttgaaccgggtaaaactattacgccgggtcaaggtttactgttattaaatcgtgatatggcaaaagccgtggcagcagtcgacgctgtagcgcatcattccttaacccagagtcagttcgatgccgtgtgcgatttagtgtataatgctggtgccggtgtgattgcggctgcgactggcacaggcaaagcactgcgctctggtgatgttgcgaccttacgtgcaaaattggcgttgttcattaaccaaaatggcaagcctctgttaggtttacgccgtcgtacggcaggacggttagccctctttgacggtaaaccgtggcaggaagcggaggccattggtcgcgccgtcaagggtctcgagcaccaccaccaccaccactga

SEQ ID NO: 13 - DNA, 672 bp, synthetic construct
  misc_feature 1..672: note = synthetic_gene encoding LNT113
  source 1..672: mol_type = other DNA
atgaaatggaaactgtttaaaaaaattgaaaaagtgggccagaacattcgcgatggcattattaaagcgggcccggcggtggcggtggtgggccaggcgacccagattgcgaaaggcggtggtggttctggtggtggcggctccggtggcggcggtagtgttagccgtaacatctcgaataacggcattaaatttacggctgcatttgagggctttcgcgggaccgcctaccgtgcaaccccaaatgaaaaatatcttaccattgggtatggcagctatggaccgcacgttgaaccgggtaaaactattacgccgggtcaaggtttactgttattaaatcgtgatatggcaaaagccgtggcagcagtcgacgctgtagcgcatcattccttaacccagagtcagttcgatgccgtgtgcgatttagtgtataatgctggtgccggtgtgattgcggctgcgactggcacaggcaaagcactgcgctctggtgatgttgcgaccttacgtgcaaaattggcgttgttcattaaccaaaatggcaagcctctgttaggtttacgccgtcgtacggcaggacggttagccctctttgacggtaaaccgtggcaggaagcggaggccattggtcgcgccgtcaagggtctcgagcaccaccaccaccaccactga